European Patent Specification EP 3 900 529 B1, published January 10, 2024. Title: Non-human animal having human IL-34 and use thereof. Applicant: Central Institute for Experimental Animals the Board of Regents of the University of Nebraska. The sequence listing filed with the application follows.

SEQUENCE LISTING (5 sequences)

SEQ ID NO: 1 - DNA, 1796 bp, Homo sapiens
  CDS (556)..(1284)
catcagacgggaagcctggactgtgggttgggggcagcctcagcctctccaacctggcacccactgcccgtggcccttaggcacctgcttggggtcctggagccccttaaggccaccagcaaatcctaggagaccgagtcttggcacgtgaacagagccagatttcacactgagcagctgcagtcggagaaatcagagaaagcgtcacccagccccagattccgaggggcctgccagggactctctcctcctgctccttggaaaggaagaccccgaaagacccccaagccaccggctcagacctgcttctgggctgccatgggacttgcggccaccgccccccggctgtcctccacgctgccgggcagataagggcagctgctgcccttggggcacctgctcactcccgcagcccagccactcctccagggccagcccttccctgactgagtgaccacctctgctgccccgaggccatgtaggccgtgcttaggcctctgtggacacactgctggggacggcgcctgagctctcagggggacgaggaacaccaccatgccccggggcttcacctggctgcgctatcttgggatcttccttggcgtggccttggggaatgagcctttggagatgtggcccttgacgcagaatgaggagtgcactgtcacgggttttctgcgggacaagctgcagtacaggagccgacttcagtacatgaaacactacttccccatcaactacaagatcagtgtgccttacgagggggtgttcagaatcgccaacgtcaccaggctgcagagggcccaggtgagcgagcgggagctgcggtatctgtgggtcttggtgagcctcagtgccactgagtcggtgcaggacgtgctgctcgagggccacccatcctggaagtacctgcaggaggtggagacgctgctgctgaatgtccagcagggcctcacggatgtggaggtcagccccaaggtggaatccgtgttgtccctcttgaatgccccagggccaaacctgaagctggtgcggcccaaagccctgctggacaactgcttccgggtcatggagctgctgtactgctcctgctgtaaacaaagctccgtcctaaactggcaggactgtgaggtgccaagtcctcagtcttgcagcccagagccctcattgcagtatgcggccacccagctgtaccctccgcccccgtggtcccccagctccccgcctcactccacgggctcggtgaggccggtcagggcacagggcgagggcctcttgccctgagcaccctggatggtgactgcggataggggcagccagaccagctcccacaggagttcaactgggtctgagacttcaaggggtggtggtgggagccccccttgggagaggacccctgggaagggtgtttttcctttgagggggattctgtgccacagcagggctcagcttcctgccttccatagctgtcatggcctcacctggagcggaggggacctggggacctgaaggtggatggggacacagctcctggcttctcctggtgctgccctcactgtccccccgcctaaagggggtactgagcctcctgtggcccgcagcagtgagggcacagctgtgggttgcaggggagacagccagcacggcgtggccattctatgaccccccagcctggcagactggggagctgggggcagagggcggtgccaagtgccacatcttgccatagtggatgctcttccagtttcttttttctattaaacaccccacttcctttggaaaaaaaaaaaaaaaaa

SEQ ID NO: 2 - protein, 242 aa, Homo sapiens
MPRGFTWLRYLGIFLGVALGNEPLEMWPLTQNEECTVTGFLRDKLQYRSRLQYMKHYFPINYKISVPYEGVFRIANVTRLQRAQVSERELRYLWVLVSLSATESVQDVLLEGHPSWKYLQEVETLLLNVQQGLTDVEVSPKVESVLSLLNAPGPNLKLVRPKALLDNCFRVMELLYCSCCKQSSVLNWQDCEVPSPQSCSPEPSLQYAATQLYPPPPWSPSSPPHSTGSVRPVRAQGEGLLP

SEQ ID NO: 3 - DNA, 20 bp, Artificial Sequence
  antisense primer for HIV-1
atctggcctggtgcaatagg

SEQ ID NO: 4 - DNA, 22 bp, Artificial Sequence
  sense primer for HIV-1
acatcaagcagccatgcaaaat

SEQ ID NO: 5 - DNA, 31 bp, Artificial Sequence
  TaqMan probe
catcaatgaggaagctgcagaatgggataga